European Patent Application EP 4 180 448 A1, published May 17, 2023. Title: Low Molecular Weight Silk Compositions and Stabilizing Silk Compositions. Applicant: Trustees of Tufts College. The sequence listing filed with the application follows.

SEQUENCE LISTING (24 sequences)

SEQ ID NO: 1 - protein, 90 aa, synthetic construct
  REGION 1..90: note = Description of Artificial Sequence: Synthetic polypeptide
  REGION 1..90: note = MISC_FEATURE - This sequence may encompass 5-15 'Gly Ala Gly Ala Gly Ser' repeating units, wherein some positions may be absent
  REGION 1..90: note = See specification as filed for detailed description of substitutions and preferred embodiments
GAGAGSGAGAGSGAGAGSGAGAGSGAGAGSGAGAGSGAGAGSGAGAGSGAGAGSGAGAGSGAGAGSGAGAGSGAGAGSGAGAGSGAGAGS

SEQ ID NO: 2 - protein, 30 aa, synthetic construct
  REGION 1..30: note = Description of Artificial Sequence: Synthetic polypeptide
  MOD_RES 2: note = Val, Ile or Ala
  MOD_RES 4: note = Val, Ile or Ala
  MOD_RES 6: note = Val, Ile or Ala
  MOD_RES 8: note = Val, Ile or Ala
  MOD_RES 10: note = Val, Ile or Ala
  MOD_RES 12: note = Val, Ile or Ala
  MOD_RES 14: note = Val, Ile or Ala
  MOD_RES 16: note = Val, Ile or Ala
  MOD_RES 18: note = Val, Ile or Ala
  MOD_RES 20: note = Val, Ile or Ala
  MOD_RES 22: note = Val, Ile or Ala
  MOD_RES 24: note = Val, Ile or Ala
  MOD_RES 26: note = Val, Ile or Ala
  MOD_RES 28: note = Val, Ile or Ala
  MOD_RES 30: note = Val, Ile or Ala
  REGION 1..30: note = MISC_FEATURE - This sequence may encompass 5-15 'Gly Xaa' repeating units, wherein some positions maybe absent
  REGION 1..30: note = See specification as filed for detailed description ofsubstitutions and preferred embodiments
GXGXGXGXGXGXGXGXGXGXGXGXGXGXGX

SEQ ID NO: 3 - protein, 4 aa, synthetic construct
  REGION 1..4: note = Description of Artificial Sequence: Synthetic peptide
GAAS

SEQ ID NO: 4 - protein, 15 aa, synthetic construct
  REGION 1..15: note = Description of Artificial Sequence: Synthetic peptide
  MOD_RES 2: note = May or may not be present
  MOD_RES 14..15: note = May or may not be present
SSAAAAAAAAAAAAA

SEQ ID NO: 5-6 - skipped (2 entries)

SEQ ID NO: 7 - protein, 12 aa, synthetic construct
  REGION 1..12: note = Description of Artificial Sequence: Synthetic peptide
  MOD_RES 2: note = May or may not be present
  MOD_RES 3..6: note = May or may not be present
  MOD_RES 8: note = May or may not be present
  MOD_RES 10..12: note = May or may not be present
  REGION 1..12: note = MISC_FEATURE - This sequence may encompass 1-2 '(Ser)1-2 (Ala)1-4' repeating units, wherein some positions may be absent
  REGION 1..12: note = See specification as filed for detailed description ofsubstitutions and preferred embodiments
SSAAAASSAAAA

SEQ ID NO: 8 - protein, 6 aa, synthetic construct
  REGION 1..6: note = Description of Artificial Sequence: Synthetic peptide
GLGGLG

SEQ ID NO: 9 - protein, 6 aa, synthetic construct
  REGION 1..6: note = Description of Artificial Sequence: Synthetic peptide
  MOD_RES 2: note = Leu, Ile, Val or Pro
  MOD_RES 5: note = Leu, Ile, Val or Pro
GXGGXG

SEQ ID NO: 10 - protein, 300 aa, synthetic construct
  REGION 1..300: note = Description of Artificial Sequence: Synthetic polypeptide
  REGION 3..14: note = MISC_FEATURE - This region may encompass 1-4 'Gly Gly Xaa' repeating units, wherein some positions may be absent
  MOD_RES 5: note = Tyr, Val, Ser or Ala
  MOD_RES 8: note = Tyr, Val, Ser or Ala
  MOD_RES 11: note = Tyr, Val, Ser or Ala
  MOD_RES 14: note = Tyr, Val, Ser or Ala
  REGION 18..29: note = MISC_FEATURE - This region may encompass 1-4 'Gly Gly Xaa' repeating units, wherein some positions may be absent
  MOD_RES 20: note = Tyr, Val, Ser or Ala
  MOD_RES 23: note = Tyr, Val, Ser or Ala
  MOD_RES 26: note = Tyr, Val, Ser or Ala
  MOD_RES 29: note = Tyr, Val, Ser or Ala
  REGION 33..44: note = MISC_FEATURE - This region may encompass 1-4 'Gly Gly Xaa' repeating units, wherein some positions may be absent
  MOD_RES 35: note = Tyr, Val, Ser or Ala
  MOD_RES 38: note = Tyr, Val, Ser or Ala
  MOD_RES 41: note = Tyr, Val, Ser or Ala
  MOD_RES 44: note = Tyr, Val, Ser or Ala
  REGION 48..59: note = MISC_FEATURE - This region may encompass 1-4 'Gly Gly Xaa' repeating units, wherein some positions may be absent
  MOD_RES 50: note = Tyr, Val, Ser or Ala
  MOD_RES 53: note = Tyr, Val, Ser or Ala
  MOD_RES 56: note = Tyr, Val, Ser or Ala
  MOD_RES 59: note = Tyr, Val, Ser or Ala
  REGION 63..74: note = MISC_FEATURE - This region may encompass 1-4 'Gly Gly Xaa' repeating units, wherein some positions may be absent
  MOD_RES 65: note = Tyr, Val, Ser or Ala
  MOD_RES 68: note = Tyr, Val, Ser or Ala
  MOD_RES 71: note = Tyr, Val, Ser or Ala
  MOD_RES 74: note = Tyr, Val, Ser or Ala
  REGION 78..89: note = MISC_FEATURE - This region may encompass 1-4 'Gly Gly Xaa' repeating units, wherein some positions may be absent
  MOD_RES 80: note = Tyr, Val, Ser or Ala
  MOD_RES 83: note = Tyr, Val, Ser or Ala
  MOD_RES 86: note = Tyr, Val, Ser or Ala
  MOD_RES 89: note = Tyr, Val, Ser or Ala
  REGION 93..104: note = MISC_FEATURE - This region may encompass 1-4 'Gly Gly Xaa' repeating units, wherein some positions may be absent
  MOD_RES 95: note = Tyr, Val, Ser or Ala
  MOD_RES 98: note = Tyr, Val, Ser or Ala
  MOD_RES 101: note = Tyr, Val, Ser or Ala
  MOD_RES 104: note = Tyr, Val, Ser or Ala
  REGION 108..119: note = MISC_FEATURE - This region may encompass 1-4 'Gly Gly Xaa' repeating units, wherein some positions may be absent
  MOD_RES 110: note = Tyr, Val, Ser or Ala
  MOD_RES 113: note = Tyr, Val, Ser or Ala
  MOD_RES 116: note = Tyr, Val, Ser or Ala
  MOD_RES 119: note = Tyr, Val, Ser or Ala
  REGION 123..134: note = MISC_FEATURE - This region may encompass 1-4 'Gly Gly Xaa' repeating units, wherein some positions may be absent
  MOD_RES 125: note = Tyr, Val, Ser or Ala
  MOD_RES 128: note = Tyr, Val, Ser or Ala
  MOD_RES 131: note = Tyr, Val, Ser or Ala
  MOD_RES 134: note = Tyr, Val, Ser or Ala
  REGION 138..149: note = MISC_FEATURE - This region may encompass 1-4 'Gly Gly Xaa' repeating units, wherein some positions may be absent
  MOD_RES 140: note = Tyr, Val, Ser or Ala
  MOD_RES 143: note = Tyr, Val, Ser or Ala
  MOD_RES 146: note = Tyr, Val, Ser or Ala
  MOD_RES 149: note = Tyr, Val, Ser or Ala
  REGION 153..164: note = MISC_FEATURE - This region may encompass 1-4 'Gly Gly Xaa' repeating units, wherein some positions may be absent
  MOD_RES 155: note = Tyr, Val, Ser or Ala
  MOD_RES 158: note = Tyr, Val, Ser or Ala
  MOD_RES 161: note = Tyr, Val, Ser or Ala
  MOD_RES 164: note = Tyr, Val, Ser or Ala
  REGION 168..179: note = MISC_FEATURE - This region may encompass 1-4 'Gly Gly Xaa' repeating units, wherein some positions may be absent
  MOD_RES 170: note = Tyr, Val, Ser or Ala
  MOD_RES 173: note = Tyr, Val, Ser or Ala
  MOD_RES 176: note = Tyr, Val, Ser or Ala
  MOD_RES 179: note = Tyr, Val, Ser or Ala
  REGION 183..194: note = MISC_FEATURE - This region may encompass 1-4 'Gly Gly Xaa' repeating units, wherein some positions may be absent
  MOD_RES 185: note = Tyr, Val, Ser or Ala
  MOD_RES 188: note = Tyr, Val, Ser or Ala
  MOD_RES 191: note = Tyr, Val, Ser or Ala
  MOD_RES 194: note = Tyr, Val, Ser or Ala
  REGION 198..209: note = MISC_FEATURE - This region may encompass 1-4 'Gly Gly Xaa' repeating units, wherein some positions may be absent
  MOD_RES 200: note = Tyr, Val, Ser or Ala
  MOD_RES 203: note = Tyr, Val, Ser or Ala
  MOD_RES 206: note = Tyr, Val, Ser or Ala
  MOD_RES 209: note = Tyr, Val, Ser or Ala
  REGION 213..224: note = MISC_FEATURE - This region may encompass 1-4 'Gly Gly Xaa' repeating units, wherein some positions may be absent
  MOD_RES 215: note = Tyr, Val, Ser or Ala
  MOD_RES 218: note = Tyr, Val, Ser or Ala
  MOD_RES 221: note = Tyr, Val, Ser or Ala
  MOD_RES 224: note = Tyr, Val, Ser or Ala
  REGION 228..239: note = MISC_FEATURE - This region may encompass 1-4 'Gly Gly Xaa' repeating units, wherein some positions may be absent
  MOD_RES 230: note = Tyr, Val, Ser or Ala
  MOD_RES 233: note = Tyr, Val, Ser or Ala
  MOD_RES 236: note = Tyr, Val, Ser or Ala
  MOD_RES 239: note = Tyr, Val, Ser or Ala
  REGION 243..254: note = MISC_FEATURE - This region may encompass 1-4 'Gly Gly Xaa' repeating units, wherein some positions may be absent
  MOD_RES 245: note = Tyr, Val, Ser or Ala
  MOD_RES 248: note = Tyr, Val, Ser or Ala
  MOD_RES 251: note = Tyr, Val, Ser or Ala
  MOD_RES 254: note = Tyr, Val, Ser or Ala
  REGION 258..269: note = MISC_FEATURE - This region may encompass 1-4 'Gly Gly Xaa' repeating units, wherein some positions may be absent
  MOD_RES 260: note = Tyr, Val, Ser or Ala
  MOD_RES 263: note = Tyr, Val, Ser or Ala
  MOD_RES 266: note = Tyr, Val, Ser or Ala
  MOD_RES 269: note = Tyr, Val, Ser or Ala
  REGION 273..284: note = MISC_FEATURE - This region may encompass 1-4 'Gly Gly Xaa' repeating units, wherein some positions may be absent
  MOD_RES 275: note = Tyr, Val, Ser or Ala
  MOD_RES 278: note = Tyr, Val, Ser or Ala
  MOD_RES 281: note = Tyr, Val, Ser or Ala
  MOD_RES 284: note = Tyr, Val, Ser or Ala
  REGION 288..299: note = MISC_FEATURE - This region may encompass 1-4 'Gly Gly Xaa' repeating units, wherein some positions may be absent
  MOD_RES 290: note = Tyr, Val, Ser or Ala
  MOD_RES 293: note = Tyr, Val, Ser or Ala
  MOD_RES 296: note = Tyr, Val, Ser or Ala
  MOD_RES 299: note = Tyr, Val, Ser or Ala
  REGION 1..300: note = MISC_FEATURE - This sequence may encompass 3-20 'Gly Pro (Gly Gly Xaa)1-4 Tyr)' repeating units, wherein some positions may be absent
  REGION 1..300: note = See specification as filed for detailed description of substitutions and preferred embodiments
GPGGXGGXGGXGGXYGPGGXGGXGGXGGXYGPGGXGGXGGXGGXYGPGGXGGXGGXGGXYGPGGXGGXGGXGGXYGPGGXGGXGGXGGXYGPGGXGGXGGXGGXYGPGGXGGXGGXGGXYGPGGXGGXGGXGGXYGPGGXGGXGGXGGXYGPGGXGGXGGXGGXYGPGGXGGXGGXGGXYGPGGXGGXGGXGGXYGPGGXGGXGGXGGXYGPGGXGGXGGXGGXYGPGGXGGXGGXGGXYGPGGXGGXGGXGGXYGPGGXGGXGGXGGXYGPGGXGGXGGXGGXYGPGGXGGXGGXGGXY

SEQ ID NO: 11 - protein, 24 aa, synthetic construct
  REGION 1..24: note = Description of Artificial Sequence: Synthetic peptide
  MOD_RES 8..24: note = May or may not be present
GRGGAAAAAAAAAAAAAAAAAAAA

SEQ ID NO: 12 - protein, 13 aa, synthetic construct
  REGION 1..13: note = Description of Artificial Sequence: Synthetic peptide
  MOD_RES 10: note = May or may not be present
GAGAAAAAAAGGA

SEQ ID NO: 13 - protein, 8 aa, synthetic construct
  REGION 1..8: note = Description of Artificial Sequence: Synthetic peptide
  MOD_RES 3: note = Gln, Tyr, Leu, Ala, Ser or Arg
  MOD_RES 5: note = Gln, Tyr, Leu, Ala, Ser or Arg
  MOD_RES 7..8: note = Gln, Tyr, Leu, Ala, Ser or Arg
GGXGXGXX

SEQ ID NO: 14 - protein, 16 aa, synthetic construct
  REGION 1..16: note = Description of Artificial Sequence: Synthetic peptide
TGSSGFGPYVNGGYSG

SEQ ID NO: 15 - protein, 8 aa, synthetic construct
  REGION 1..8: note = Description of Artificial Sequence: Synthetic peptide
YEYAWSSE

SEQ ID NO: 16 - protein, 7 aa, synthetic construct
  REGION 1..7: note = Description of Artificial Sequence: Synthetic peptide
SDFGTGS

SEQ ID NO: 17 - protein, 7 aa, synthetic construct
  REGION 1..7: note = Description of Artificial Sequence: Synthetic peptide
RRAGYDR

SEQ ID NO: 18 - protein, 8 aa, synthetic construct
  REGION 1..8: note = Description of Artificial Sequence: Synthetic peptide
EVIVIDDR

SEQ ID NO: 19 - protein, 18 aa, synthetic construct
  REGION 1..18: note = Description of Artificial Sequence: Synthetic peptide
TTIIEDLDITIDGADGPI

SEQ ID NO: 20 - protein, 8 aa, synthetic construct
  REGION 1..8: note = Description of Artificial Sequence: Synthetic peptide
TISEELTI

SEQ ID NO: 21-24 - skipped (4 entries)